European Patent Specification EP 3 377 106 B1, published May 24, 2023. Title: Modulation of ciliogenesis. Applicant: Academisch Ziekenhuis Leiden a/u leiden University Medical Center Van Brempt, Ronald. The sequence listing filed with the application follows.

SEQUENCE LISTING (25 sequences)

SEQ ID NO: 1 - DNA, 425 bp, Mus musculus
acactgacacggaccgaaggagtggaaaaagctttacctgtcactgtctgctgccatacgatgctgggaggcctggggaagctggcggccgagggcctggcccaccgcacagagaaagccactgggggagcagttcacgcagtggaagaggtggtgagcgaggtggtgggccacgccaaggaggttggagagaagaccattaatgacgccctaaagaaagcccaagaatcaggagacagggtggtgaaggaggtcactgagaaggtcacccacaccatcactgatgctgttacccatgcggcagaaggcctgggaagactgggacagtgagcctgcctaccagcatggctggcccttcctgaaggtcaataaagagtgtgaaacgtgaaaaaaaaaaaaaaaataacaaaaaaaaaaaaaaaaaa

SEQ ID NO: 2 - DNA, 267 bp, Mus musculus
atgctgggaggcctggggaagctggcggccgagggcctggcccaccgcacagagaaagccactgggggagcagttcacgcagtggaagaggtggtgagcgaggtggtgggccacgccaaggaggttggagagaagaccattaatgacgccctaaagaaagcccaagaatcaggagacagggtggtgaaggaggtcactgagaaggtcacccacaccatcactgatgctgttacccatgcggcagaaggcctgggaagactgggacag

SEQ ID NO: 3 - DNA, 342 bp, Homo sapiens
actgtctgctgccacacgatgctgggaggcctggggaagctggctgccgaaggcctggcccaccgcaccgagaaggccaccgagggagccattcatgccgtggaagaagtggtgaaggaggtggtgggacacgccaaggagactggagagaaagccattgctgaagccataaagaaagcccaagagtcaggggacaaaaagatgaaggaaatcactgagacagtgaccaacacagtcacaaatgccatcacccatgcagcagagagtctggacaaacttggacagtgagtgcacctgctaccacggcccttccccagtctcaataaaaagccatgacatgtg

SEQ ID NO: 4 - DNA, 267 bp, Homo sapiens
atgctgggaggcctggggaagctggctgccgaaggcctggcccaccgcaccgagaaggccaccgagggagccattcatgccgtggaagaagtggtgaaggaggtggtgggacacgccaaggagactggagagaaagccattgctgaagccataaagaaagcccaagagtcaggggacaaaaagatgaaggaaatcactgagacagtgaccaacacagtcacaaatgccatcacccatgcagcagagagtctggacaaacttggacag

SEQ ID NO: 5 - protein, 89 aa, Mus musculus
MLGGLGKLAAEGLAHRTEKATGGAVHAVEEVVSEVVGHAKEVGEKTINDALKKAQESGDRVVKEVTEKVTHTITDAVTHAAEGLGRLGQ

SEQ ID NO: 6 - protein, 89 aa, Homo sapiens
MLGGLGKLAAEGLAHRTEKATEGAIHAVEEVVKEVVGHAKETGEKAIAEAIKKAQESGDKKMKEITETVTNTVTNAITHAAESLDKLGQ

SEQ ID NO: 7 - DNA, 200 bp, Homo sapiens
gttccccagcatcctcggctcctgcctcactagctgcggagcctctcccgctcggtccacgctgccgggcggccacgaccgtgacccttcccctcgggccgcccagatccatgcctcgtcccacgggacaccagttccctggcgtgtgcagaccccccggcgcctaccatgctgtacgtcggtgaccccgcacggcacct

SEQ ID NO: 8 - DNA, 200 bp, Homo sapiens
gcggaggcagagcggccctggggccccggcgtcagctgaggttgcactgtgtttggagaggagcctcggaggggtgggctgcctggcagcagtggcctgggggccgcaaatgaggagggtgcagtgccttgggcagtaaattagaagacacaggctgctggctgggggcgggagggcacagggaagccctgcccgggagc

SEQ ID NO: 9 - DNA, 200 bp, Homo sapiens
cgggacttcctgacgcccccgctgctgtccgtgcgcttccggtgagtcaggtacggcgcggccggtgggcggagcctccggggtgaggggcggggcctaatggagcctccctttcacctcatcaggtacggtggcgccccccaggccctcaccctgaagctcccagtgaccatcaacaagttcttccagcccaccgagat

SEQ ID NO: 10 - DNA, 200 bp, Homo sapiens
atcctagggaggggcacctctcgagggggtttctgggagagggcagtggaacctggccccgctgacacccactcctgcacacagccccccagtgcagttctccctgctccactccaagttccatctgtgcagcgtggccacgcgggcgctgctgctgtccacctacatcaagttcatcaacctcttccccgagaccaagg

SEQ ID NO: 11 - DNA, 294 bp, Homo sapiens
cccagggaggtgagggctcagagggtggcgagggcacataggaggggagcggaagcctggctctcaggcctaggcccctatcctgccccaggccaggtccaggccctggaccccgcctagcgtaggctagtgtgtatccctggaaccagaagagagtaggtggctctggaggcctctcaggcccccccagactctgtgaccccccacaccccaggacatgcgtgggcgctatgaggcaagccaggacctactgggcaccctgcggaagcagcttagcgacagcgagagcgagcg

SEQ ID NO: 12 - DNA, 258 bp, Homo sapiens
tccagggactggctgtgcatactggcagatgtcagtcagccctcctgcagttgggccagggacacctcagggaaactgtgaccttccttccaatcttggtaacatcacccttccaccccaaatcccagggaatggcccgaatctctcctgacaaacagctctcagccctggtccaggccacagtcttgcttgcaccgggccgggtttcagagcccgaagggcacactggcagcctttagtgcagtgtttcagatgtca

SEQ ID NO: 13 - DNA, 200 bp, Homo sapiens
gtggcgcacacggtgtagttatgtggcttgaggatctgggaaaggcacactcagttgcagctggtgtgctggcgtgtggcgttttggtgctctaaccattgtctgtgttcaactcccaagctacagacgggccccctccttgggagcgccagggatgttggcgccctggagccccagacagggagagactcagagggccc

SEQ ID NO: 14 - DNA, 262 bp, Homo sapiens
cgactacagggaatggaaatggtatagccatcatctaaaaaccatctcccgggttggaaacccaccagcatttcccttcctggttctgtctggctcaggtgtacatggacaggaaaattaatttccatgacccaagtaggtgcttagttaatgttagatgagcagaaagaagccctgagttcagagattcgatggggaacggtgcagggaagtggggctcggattctggggccaagagagtcatctgaaaaccacagagaac

SEQ ID NO: 15 - DNA, 200 bp, Homo sapiens
aggggaccccgaccggcggagggacggctgcgccctgcaggccgctgcgcccaggcaggcctctgcgcccgggcaggcctcggcctcctgtcgcgcccccggcccgcgacaatccgggcaggatgggcggcaggacgcggaggggcatctgcggagcccgtcgggaacgccctcttggcttccggtgccgggcagcggcg

SEQ ID NO: 16 - DNA, 200 bp, Homo sapiens
tgcgccctgcaaccccctcccttgcccgggcccccctcacctgcgcgggccgggggcgcagccgcgaagcctgcctggcgcgcggggcctgcagattcggccggcggggaggggatgcggaaccagtcgcgcccaaacctcgggtcggcgacctggcgccccgccacccccaacactgccccgaggcccggtgacaatga

SEQ ID NO: 17 - DNA, 200 bp, Homo sapiens
gttgggtggcgttgggggagctgcgcctcgcccagagcctcgcccggagcctcgcccggagccttccggggtgggggatagttgaggacctcatcgagggaggggttgggcggcggggaagggagcgagcgtggcgggggacccgaggcacgctctcgagccaacgagcgtgatgcgctcgagtgtgggcggggactgag

SEQ ID NO: 18 - DNA, 287 bp, Homo sapiens
aagccccgggtcccaggcgggcagagggtgggggtggcggcgccgcgcggagcacccgggaagcgcccccttcgcggtccagccccgcacccccgccccgcggcgggcggcgcccgagtcctcgccgcaaacccgaggagcaggatgtggaaagcagccgcggcggtggctgcggctgcggcgcctacaccgagcagccgatcgcatcacttaccccttaccgtggagagagggaccggacgggggaggcggggcgcgtcgcgtcccgtgagtctctcgcacgccgt

SEQ ID NO: 19 - DNA, 290 bp, Homo sapiens
cgctctgccgtgggctcggcccgggctgccacgagcgtgcgggcctcgccgggcatgtcctaggcggcggccccgcccagcgctcggccgggcgggcgggcgggcgcgagggcagggaccgagccgggccgagctggggaacaagccggggaccaagccggggaccaagccggggactaaggcgagccggagaccgagcccgaacagcaggtaggacgcgccggcccagcgctggccgcggcccgggcctcccatcgcccgcacctgcacggctgtggggtctcacgggg

SEQ ID NO: 20 - DNA, 200 bp, Homo sapiens
agaccttgggcgtgggcactgggcaaagtagggacaaggagccactcactcctctgcctggcaccctcatgtggtgtggccctgccctcaggatgcactcagcccggcagcctccccttctcctctgctccactgggcctcagctgctgtcatccctgtcctgggttattgtcctcacttcttgactggcctcctgagtc

SEQ ID NO: 21 - DNA, 200 bp, Homo sapiens
gggccgcggcaggtgatggcagagggtgaggcctaggagggctggctgggggccggaggtgcaatggtggggtaggccctgcccgatagagcaccctgtggtctcccccagcagccctagggagggtggggctgtagaggcctcctggaggctttgctgtctggggctgcagggtcatcgaagtgccagccccttggcct

SEQ ID NO: 22 - DNA, 200 bp, Homo sapiens
tggtgtttcatgacggtgccctgtggtggggcagtgatggccagctgccagggtggcctgcacgtggcaggctaagagtgaccagcctgaggggcccaggctctcacctgggagactgagaagccgtgctggcactcaggagggacttccagctcctagtcgtgtgggttgcaggccgtcctgtcccagggctgggggac

SEQ ID NO: 23 - DNA, 200 bp, Homo sapiens
gaagtcggggacgcgggctcggtgaggggggacgctggtgcctcggcctgcgcctaggcgggaggcagacgcatgcacctttggcctacgtttcggctgccggaccgacgggacagtgacggttgggccgggtgggggcgcaggctgtggggcggcctcagggcgcgagcaaggggactgccgcgcttcccgcgcctctg

SEQ ID NO: 24 - DNA, 200 bp, Homo sapiens
ttggcccagcggcacgcgaagcaggaagtcccaccccccacgccgacgtcacccacgccaccgacgccggttgctgccggagccgttagagggaggagacaaacgaaccgaggcgggagcggccacgggtgacagcggcagcggcggggccgggctgcgctcccgaaggcgttcctggagggccctgggatggactcaga

SEQ ID NO: 25 - DNA, 199 bp, Homo sapiens
accgacgggacagcggcatctcctccacctgaaaaggaaagaggaccaggtgggggccaggcagggcgcatgaaggcggcgccagcaccgcgcgatccgaatcacgtcggtgcgggggaggggtcggagcctggcctcggcctagggcgcagatgcggtgcgcaccgcaggggggcggcgtggggtgcggggccagtcc